European Patent Specification EP 4 015 652 B1, published August 6, 2025. Title: COMPANION METHODS AND KITS FOR IL-2-BASED THERAPIES AND MESENCHYMAL STEM CELL-BASED THERAPIES. Applicant: LUNYAK, Victoria GAUR, Meenakshi. Application PCT/US2016/035472. The sequence listing filed with the application follows.

SEQUENCE LISTING (12 sequences)

SEQ ID NO: 1 - DNA, 19 bp, Artificial Sequence
  Synthetic Construct
ctgccactcggaacacaac

SEQ ID NO: 2 - DNA, 18 bp, Artificial Sequence
  Synthetic Construct
tggtccactggctgcatt

SEQ ID NO: 3 - DNA, 20 bp, Artificial Sequence
  Synthetic Construct
actcgagagccaacatctcc

SEQ ID NO: 4 - DNA, 19 bp, Artificial Sequence
  Synthetic Construct
tccgaggatcaggttgcag

SEQ ID NO: 5 - DNA, 19 bp, Artificial Sequence
  Synthetic Construct
tggatgggcagaaacgcta

SEQ ID NO: 6 - DNA, 20 bp, Artificial Sequence
  Synthetic Construct
ggcttccaatgcaaacagga

SEQ ID NO: 7 - DNA, 20 bp, Artificial Sequence
  Synthetic Construct
acgcaggacacagagaatga

SEQ ID NO: 8 - DNA, 19 bp, Artificial Sequence
  Synthetic Construct
ctgggcaaactgagcttgg

SEQ ID NO: 9 - DNA, 19 bp, Artificial Sequence
  Synthetic Construct
acacagctccagaacacgt

SEQ ID NO: 10 - DNA, 19 bp, Artificial Sequence
  Synthetic Construct
tgttggcttctcggaccaa

SEQ ID NO: 11 - DNA, 20 bp, Artificial Sequence
  Synthetic Construct
ggaggagggcagaatcatca

SEQ ID NO: 12 - DNA, 19 bp, Artificial Sequence
  Synthetic Construct
atcaggggcacacaggatg